European Patent Specification EP 4 058 584 B1, published July 1, 2026. Title: GENE DELIVERY SYSTEMS FOR TREATMENT OF HEART FAILURE. Applicant: Icahn School of Medicine at Mount Sinai. The sequence listing filed with the application follows.

SEQUENCE LISTING (37 sequences)

SEQ ID NO: 1 - DNA, 1265 bp, Artificial Sequence
  Synthesized Sequence
atggcgtcctcctcggtcccaccagccacggtatcggcggcgacagcaggccccggcccaggtttcggcttcgcctccaagaccaagaagaagcatttcgtgcagcagaaggtgaaggtgttccgggcggccgacccgctggtgggtgtgttcctgtggggcgtagcccactcgatcaatgagctcagccaggtgcctcccccggtgatgctgctgccagatgactttaaggccagctccaagatcaaggtcaacaatcaccttttccacagggaaaatctgcccagtcatttcaagttcaaggagtattgtccccaggtcttcaggaacctccgtgatcgatttggcattgatgaccaagattacttggtgtcccttacccgaaacccccccagcgaaagtgaaggcagtgatggtcgcttccttatctcctacgatcggactctggtcatcaaagaagtatccagtgaggacattgctgacatgcatagcaacctctccaactatcaccagtacattgtgaagtgccatggcaacacgcttctgccccagttcctggggatgtaccgagtcagtgtggacaacgaagacagctacatgcttgtgatgcgcaatatgtttagccaccgtcttcctgtgcacaggaagtatgacctcaagggttccctagtgtcccgggaagccagcgataaggaaaaggttaaagaattgcccacccttaaggatatggactttctcaacaagaaccagaaagtatatattggtgaagaggagaagaaaatatttctggagaagctgaagagagatgtggagtttctagtgcagctgaagatcatggactacagccttctgctaggcatccacgacatcattcggggctctgaaccagaggaggaagcgcccgtgcgggaggatgagtcagaggtggatggggactgcagcctgactggacctcctgctctggtgggctcctatggcacctccccagagggtatcggaggctacatccattcccatcggcccctgggcccaggagagtttgagtccttcattgatgtctatgccatccggagtgctgaaggagccccccagaaggaggtctacttcatgggcctcattgatatccttacacagtatgatgctaagaagaaagcagctcatgcagccaaaactgtcaagcatggggctggggcagagatctctactgtccatccggagcagtatgctaagcgattcctggattttattaccaacatctttgccta

SEQ ID NO: 2 - DNA, 20 bp, Artificial Sequence
  Synthesized Sequence
ggagactatggcgtcctcct

SEQ ID NO: 3 - DNA, 20 bp, Artificial Sequence
  Synthesized Sequence
ccggaacaccttcactttct

SEQ ID NO: 4 - DNA, 21 bp, Artificial Sequence
  Synthesized Sequence
agtccctgccctttgtacaca

SEQ ID NO: 5 - DNA, 18 bp, Artificial Sequence
  Synthesized Sequence
gatccgagggcctcacta

SEQ ID NO: 6 - DNA, 21 bp, Artificial Sequence
  Synthesized Sequence
aggaagccgaggttttaactg

SEQ ID NO: 7 - DNA, 21 bp, Artificial Sequence
  Synthesized Sequence
aggacgctcataagtgtcacc

SEQ ID NO: 8 - DNA, 19 bp, Artificial Sequence
  Synthesized Sequence
ctggcaagaagggagatga

SEQ ID NO: 9 - DNA, 20 bp, Artificial Sequence
  Synthesized Sequence
caccatccaaaccactgaaa

SEQ ID NO: 10 - DNA, 20 bp, Artificial Sequence
  Synthesized Sequence
aggtcttcctggagctgatg

SEQ ID NO: 11 - DNA, 20 bp, Artificial Sequence
  Synthesized Sequence
ccccacagggccttctttac

SEQ ID NO: 12 - DNA, 20 bp, Artificial Sequence
  Synthesized Sequence
gtggggtagagagtgggtca

SEQ ID NO: 13 - DNA, 20 bp, Artificial Sequence
  Synthesized Sequence
tgctgtgcccagatgtagag

SEQ ID NO: 14 - DNA, 24 bp, Artificial Sequence
  Synthesized Sequence
acagcaaattcacttacacagttc

SEQ ID NO: 15 - DNA, 19 bp, Artificial Sequence
  Synthesized Sequence
ctcattgccttgcgtgttt

SEQ ID NO: 16 - DNA, 21 bp, Artificial Sequence
  Synthesized Sequence
aggaagccgaggttttaactg

SEQ ID NO: 17 - DNA, 21 bp, Artificial Sequence
  Synthesized Sequence
aggaagccgaggttttaactg

SEQ ID NO: 18 - DNA, 20 bp, Artificial Sequence
  Synthesized Sequence
cagaacaccagcctcatcaa

SEQ ID NO: 19 - DNA, 20 bp, Artificial Sequence
  Synthesized Sequence
gctccttcttcagctcctca

SEQ ID NO: 20 - DNA, 19 bp, Artificial Sequence
  Synthesized Sequence
gcttccaggcatattggag

SEQ ID NO: 21 - DNA, 19 bp, Artificial Sequence
  Synthesized Sequence
gggggcatgacctcatctt

SEQ ID NO: 22 - DNA, 18 bp, Artificial Sequence
  Synthesized Sequence
aagggtctggctgctttg

SEQ ID NO: 23 - DNA, 22 bp, Artificial Sequence
  Synthesized Sequence
cagccaggacttcctcttaatg

SEQ ID NO: 24 - DNA, 21 bp, Artificial Sequence
  Synthesized Sequence
aggacgctcataagtgtcacc

SEQ ID NO: 25 - DNA, 21 bp, Artificial Sequence
  Synthesized Sequence
aggaagccgaggttttaactg

SEQ ID NO: 26 - DNA, 20 bp, Artificial Sequence
  Synthesized Sequence
gctgccatttctaataaaga

SEQ ID NO: 27 - DNA, 18 bp, Artificial Sequence
  Synthesized Sequence
gcacttcctttcacaaag

SEQ ID NO: 28 - DNA, 20 bp, Artificial Sequence
  Synthesized Sequence
ttgaaggatggcaagtatgg

SEQ ID NO: 29 - DNA, 21 bp, Artificial Sequence
  Synthesized Sequence
cgaaggcatgacctagagtgt

SEQ ID NO: 30 - DNA, 27 bp, Artificial Sequence
  Synthesized Sequence
aaggacggccttctggcacacgccttt

SEQ ID NO: 31 - DNA, 24 bp, Artificial Sequence
  Synthesized Sequence
gtggtatagtgggacacatagtgg

SEQ ID NO: 32 - DNA, 24 bp, Artificial Sequence
  Synthesized Sequence
gagatcaaggccaatgttcggagg

SEQ ID NO: 33 - DNA, 21 bp, Artificial Sequence
  Synthesized Sequence
cggtagtacttattgcccaag

SEQ ID NO: 34 - DNA, 17 bp, Artificial Sequence
  Synthesized Sequence
cctgtccaaactaaggc

SEQ ID NO: 35 - DNA, 19 bp, Artificial Sequence
  Synthesized Sequence
ggttttctcatagatggcg

SEQ ID NO: 36 - DNA, 3354 bp, Artificial Sequence
  Synthesized Sequence
atgacggctgcgcaggtgagcaccgcttccgggtcgggcttcggagtcgcggctagctcccgcttccactcgctcgggtgcgcgggagactatggcgtcctcctccgtccctcccgccaccgcacccgcggcagctggaggccccggcccgggattcggcttcgcctccaaaaccaagaagaagcatttcgtacagcagaaagtgaaggtgttccgggccgcggacccgctggtgggcgtgttcctgtggggcgtcgctcactcgatcaatgagctcagccaggtaccgcccccagtgatgttgctgccagatgactttaaagccagctccaagatcaaggtcaacaatcactttttccatagagaaaatcttcccagtcatttcaagttcaaggagtattgtccccaggtcttcaggaacctgagagatcggtttgccatcgatgatcacgattacttggtgtcccttactcgaagccccccaagcgaaactgaaggcagtgatggccgtttccttatctcctatgaccgcactctggtcatcaaggaagtgtcgagcgaagatattgcggatatgcacagcaacctctccaactaccaccagtacatagtgaaatgtcatggcaacacgcttctgccccagttcctgggcatgtaccgagtcagtgtagaaaatgaagacagctacatgctcgtgatgcgcaatatgtttagtcatcgtcttcctgtgcataggaagtatgacctcaagggctctctagtgtcccgggaagccagcgataaggaaaaggttaaagaactgccaacactaaaggatatggactttcttaacaagaaccagaaagtgtatattggtgaagaagaaaagaaagtattcctggagaagctgaagcgagatgtggagtttctagtgcagctgaagatcatggactacagcctcctgttgggcatccacgacatcatccggggctctgaacccgaggaagaggggcctgtgagggaggaggagtctgagtgggatggggactgtaacctggctggacctcccgccctggtgggctcctatggtacctcccctgagggtatcggaggctacatccattcccaccggccactgggcccaggagagtttgagtccttcatcgatgtctatgctatccggagtgcggagggggccccccagaaggaggtgtatttcatgggcctcattgacattctgacacagtatgatgccaagaagaaagcagctcatgcagccaagactgtcaagcacggggcgggggcagagatctccactgtccatcctgagcagtatgctaagcgattcctggactttattgccaacatctttgcctaagaggctgcctgactccagggtgattgcggctttatgttggaggtggcgggttctgagaggcttaggggagctggacttggccgttacttctcttctttgctaaattcaggctgcaggctccttccatccaaataacttccttctggtggatagggttttctcgcccaccccagacatacactgtcctttctccccttgtccatttctctgccctccctccttgctcccagtaagccctcctgcttctttagagtgttattgtcgactcttctaagtgccttgatctttgaaaaatatcttgtttctatgaaataggaggagctgggggaggggttgtttgccatcttcgggacctgactgaacagtggacttggctcaagcaactgcctggatgcacttttgctgagtggaagaaactgaatgtctggattttgctgatacttttatggggcactttgtggcatgcttcctccctggtaagccctggaatggagggctttcaggatgctccagatgtgggtgcaggcattcacacatggacagtctggcctggaggtcaggtggggagtggtcagcaggctggcacctcacaaggcaggacctaagcctaagcggacttttgtgactatgcagatgatggagaaggtccctgtggagcaacgactgttcccgactgttcccgttctcccaccccaccccaccccacgtccacctctttctgtgagcactttgggtgcaggagcccagaggctagcggtgcccgagcttaggtgcaggtgtgagactcgggctgctcttcccacaaccctgtgccttgctggtgagcagggagagcagtagaggccgggacaggtcggagtgcagggttcattgcctgggtgacaccctttcttcctgtctcactactcctgggcttctttctagcagaggggaacagtaccatctccataatttggggaggatagagctctcgagtgaaggagcctccgcatccctggggcatgtgtacctagaactccccctccttctcaaaaccctttctggttggagttgttattctgtcccatcttccactgctaatgtgtctcccaggggacagatggccttctttgtcatctcccctctccgcccccagagaggagtcagagccataactcaatccacccagtcctctccaaagacagctgaatattaatgcacgccatcctcagaatggagaggacctgctaggcatcttagctctcccagctcgtgcctgtaaagccagcactcaggaggctctgagagttcaagtccagcctgggctactgagtgagacctggtctcaggaacactccaaataggtttgggtttgagcgctggagatcatagctgagttggtagtgtgcttgcctagcatgtacaaagctctgggatccacccccagcaccacttaagccaggcgtggcggtgcacgcctgcactcctggccctgggaagtagtggtaagcaggatggggcattcaaggtcatcgccagttagttacttgacgaggttgaggccagccaaggaaacaggagaccatcttggggaaaatgattctaaggagagatagattgtctttgtctctgcctaaagcctttggaagcaagccactcatcttcgctgtttggcgctctggaggtggggtgggcattgaaggcaaggagctgctttgctgtgtgtccatgaggtcctcagggagaagcccacctccctcaccaaaggaagcagcaagatgggtgcccggttggggtgggtgggacctgctgagtctcccatccctcaagcaacctttcccctgttgaatgcaataagtgactccggtcccttaacaactggggtctcaccgtgcggctgtggtcgtgggcagtgttgccatcttcacttactgcttccgttttccatctgttttgttaataaaatatgtatatttactcccgatatcacaataaaataaattatttgatctaagtca

SEQ ID NO: 37 - DNA, 1653 bp, Artificial Sequence
  Synthesized Sequence
atggccgatgctaagaacattaagaagggccctgctcccttctaccctctggaggatggcaccgctggcgagcagctgcacaaggccatgaagaggtatgccctggtgcctggcaccattgccttcaccgatgcccacattgaggtggacatcacctatgccgagtacttcgagatgtctgtgcgcctggccgaggccatgaagaggtacggcctgaacaccaaccaccgcatcgtggtgtgctctgagaactctctgcagttcttcatgccagtgctgggcgccctgttcatcggagtggccgtggcccctgctaacgacatttacaacgagcgcgagctgctgaacagcatgggcatttctcagcctaccgtggtgttcgtgtctaagaagggcctgcagaagatcctgaacgtgcagaagaagctgcctatcatccagaagatcatcatcatggactctaagaccgactaccagggcttccagagcatgtacacattcgtgacatctcatctgcctcctggcttcaacgagtacgacttcgtgccagagtctttcgacagggacaaaaccattgccctgatcatgaacagctctgggtctaccggcctgcctaagggcgtggccctgcctcatcgcaccgcctgtgtgcgcttctctcacgcccgcgaccctattttcggcaaccagatcatccccgacaccgctattctgagcgtggtgccattccaccacggcttcggcatgttcaccaccctgggctacctgatttgcggctttcgggtggtgctgatgtaccgcttcgaggaggagctgttcctgcgcagcctgcaagactacaaaattcagtctgccctgctggtgccaaccctgttcagcttcttcgctaagagcaccctgatcgacaagtacgacctgtctaacctgcacgagattgcctctggcggcgccccactgtctaaggaggtgggcgaagccgtggccaagcgctttcatctgccaggcatccgccagggctacggcctgaccgagacaaccagcgccattctgattaccccagagggcgacgacaagcctggcgccgtgggcaaggtggtgccattcttcgaggccaaggtggtggacctggacaccggcaagaccctgggagtgaaccagcgcggcgagctgtgtgtgcgcggccctatgattatgtccggctacgtgaataaccctgaggccacaaacgccctgatcgacaaggacggctggctgcactctggcgacattgcctactgggacgaggacgagcacttcttcatcgtggaccgcctgaagtctctgatcaagtacaagggctaccaggtggccccagccgagctggagtctatcctgctgcagcaccctaacattttcgacgccggagtggccggcctgcccgacgacgatgccggcgagctgcctgccgccgtcgtcgtgctggaacacggcaagaccatgaccgagaaggagatcgtggactatgtggccagccaggtgacaaccgccaagaagctgcgcggcggagtggtgttcgtggacgaggtgcccaagggcctgaccggcaagctggacgcccgcaagatccgcgagatcctgatcaaggctaagaaaggcggcaagatcgccgtgtaa